European Patent Application EP 4 471 135 A1, published December 4, 2024. Title: フルクトシルアミノ酸オキシダーゼ、フルクトシルアミノ酸オキシダーゼの製造方法、糖化タンパク質センサ、及び糖化タンパク質の測定方法。. Applicant: PROVIGATE INC. Application WO. The sequence listing filed with the application follows.

SEQUENCE LISTING (35 sequences)

SEQ ID NO: 1 - protein, 446 aa, Aspergillus pseudotamarii
MASSNLTLTSSILIVGAGTWGCSTALHLARRGYKNVTVLDPHPVPSPIAAGNDINKIMEHREVKASETDPWSIAFSTCTRAALKGWKTDPVFQPYFHETGAIVSGHTPSLIKHIEEHEIDSSDAEFVKLNTAEDFRKTMPPGILTGNFPGWKGWLNKTGAGWIHAKKAMFSAYTEAKRLGVTFITGSPEGDVVSLVYENGDVAGARTADGTIHRAEHTILSAGAGSDRLLDFKKQLRPTAWTLCHIKMTPEEAKKYRNLPVLFNVAKGFFMEPDEDKHELKICDEHPGYCNFIPDPKHGGEVRSIPFAKHQIPLEAEARARDFLRDTMPHLADRPLSFARICWDADTVDRAFLIDRHPEYRSLLLAVGGSGNGAMQMSTIGGFITDALEGHLQKELKHALRWRPEIATERDWKDTQNRFGGPNKVMDFQKVGENEWTKIGDDKCRL

SEQ ID NO: 2 - protein, 447 aa, Penicillium rubens
MATLELNHTTSILIVGAGTWGCSTALHLARRGYRNVKVLDPHPVPSPIAAGNDINKIMEHKELKSPKPDARSIAFATCTRAALKGWKTDPVFQPYFHETGFIVSGHTPALIEHIKTEEIDPSEGDWVALESAEDFRQTMPPGVLTGDFPGWKGWISRVGAGWIHARKAMVSAYNEAQRLGVDFVTGSPQGNVESLIYKDADVVGARTADGLSHYADRTILAAGAGSDRLLDFKKQLRPTAWTLSHIRMTPEEADKYRNLPVLFNVAKGFFMEPDEEKHELKICDEHPGYCNFVVDPDHQGEKRSIPFAKEQIPLEAEARARDFLRDTMPHLADRPFSFARICWDADTVDRAFLIDRHPEYASLVVAVGGSGNGAMQMPTIGGFISDTLEGKLQKELKDVVRWRPETAIHRDWKSTQNRFGGPDRLMDFQDVKDDEWTRIGEDMASRL

SEQ ID NO: 3 - protein, 447 aa, Penicillium flavigenum
MATLELNHASSILIVGAGTWGCSTALHLARRGYKNVKVLDPHPVPSPIAAGNDINKIMEHKELKSPKPDARSIAFATCTRAALKGWKTDPVFQPYFHETGFIVSGHTPALIEHIKTEDIDPSEGDWAALESAEDFRQTMPPGVLTGDFPGWKGWISRVGTGWIHARKAMVSAYNEAQRLGVSFVTGSPEGNVESLIYKDGDVVGARTADGLSHYADRTILAAGAGSDRLLDFKKQLRPTAWTLSHIRMTPEEAEKYRNLPVLFNVAKGFFMEPDEEKHELKICDEHPGYCNFVVDPDHQGEKRSIPFAKEQIPLEAEARARDFLRDTMPHLADRPFSFARICWDADTVDRAFLIDRHPEYASLVVAVGGSGNGAMQMPTIGGFISDVLEGKLQKELKDVVRWRPEIAIRRDWKSTQNRFGGPDRLMDFQDVKDDEWTSIGEEMASRL

SEQ ID NO: 4 - protein, 440 aa, Monascus purpureus
MASELSTSSSILIVGAGTWGCSTALHLARRGYKHVTVLDPYPVPSPIAAGNDVNKIMEHKEVAGIIAFATCTRAALKGWQTDPVFKPYFHETGFIQAGHTPALIEHIRQNDLYPSESDFVKLETAEDFRKTMPPGVLTGDFPGWKGWLMKKNAGWIHARKAMFSAFHEAKRLGVTFITGSPQGKVVSLVYGQDDVTGARTEDGKVHSADRVIVSAGAGTDRILDMENQLRPTAWTLCHIKMTEEEIKSQRYRNLPVLFNIAKGFFMEPDEDKGELKMCDEHPGYVNWVSDPNRPGEKRSIPFAKEQIPREAERRAREFLKDTMPHLADRPLVFARICWDADTPDRFFLIDYHPRYPSLLLACGGSGNGAMQMPSIGGFIADALEGRLQEELKDVCRWRPETAVGRDWKSTQGRFGGPDKVMDFQEVGENEWTRVGKESLL

SEQ ID NO: 5 - protein, 443 aa, Coniochaeta pulveracea
MAGGLGTQSRILILGGGTWGCSTALHLARRGYKNVTVLDAHPIPSPISAGNDVNKIVEQGCFTDGDDEAAVAQTLLHAANEGWQKDPVFQPYYHDTGYIVAGSSPKAIERLVDREVRHQASSFRKLTTAEDFKGTMPTGVLTGDFPGWEGYYKPSGAGWVHARKALVSAYNEAKRLGVNFITGSPEGKVKSLLLEDGDVRGAITADGVEHRADRTILAMGANAPQLLDFENQLRPTAWTLAHIPMTEEETRLYKNLPVLFNIEKGFFMEPDEDKHELKLCDEHPGYCNWVDQPGSALPQSVPVAKHEVPASAERRMRDFLREIMPHLADRPFTFARMCWCADTRNRAFLITYHPKHPSLVVASGDSGHGFMHIPSIGGFIVDCMENKLQPNFAKSWRWRPETTRDFWGRDVLDRFGAGNKMLDVNETREEGWTNVNATPLTVA

SEQ ID NO: 6 - protein, 447 aa, synthetic construct
MATLELNHTTSILIVGAGTWGCSTALHLARRGYRNVKVLDPHPVPSPIAAGNDINKIMEHRELKSPEPDARSIAFATCTRAALKGWKTDPVFQPYFHETGFIVSGHTPALIEHIKTEEIDPSEGDWVKLESAEDFRQTMPPGVLTGDFPGWKGWISKVGAGWIHAKKAMVSAYNEAQRLGVDFVTGSPQGNVESLIYKDADVVGARTADGLSHYADRTILAAGAGSDRLLDFKKQLRPTAWTLSHIRMTPEEADKYRNLPVLFNVAKGFFMEPDEEKHELKICDEHPGYCNFVVDPDHQGEKRSIPFAKEQIPLEAEARARDFLRDTMPHLADRPFSFARICWDADTVDRAFLIDRHPEYASLVVAVGGSGNGAMQMPTIGGFISDTLEGHLQKELKDVVRWRPETAIHRDWKSTQNRFGGPDRLMDFQDVKDDEWTRIGEDMASRL

SEQ ID NO: 7 - protein, 447 aa, synthetic construct
MATLELNHASSILIVGAGTWGCSTALHLARRGYKNVKVLDPHPVPSPIAAGNDINKIMEHRELKSPEPDARSIAFATCTRAALKGWKTDPVFQPYFHETGFIVSGHTPALIEHIKTEDIDPSEGDWAKLESAEDFRQTMPPGVLTGDFPGWKGWISKVGTGWIHAKKAMVSAYNEAQRLGVSFVTGSPEGNVESLIYKDGDVVGARTADGLSHYADRTILAAGAGSDRLLDFKKQLRPTAWTLSHIRMTPEEAEKYRNLPVLFNVAKGFFMEPDEEKHELKICDEHPGYCNFVVDPDHQGEKRSIPFAKEQIPLEAEARARDFLRDTMPHLADRPFSFARICWDADTVDRAFLIDRHPEYASLVVAVGGSGNGAMQMPTIGGFISDVLEGHLQKELKDVVRWRPEIAIRRDWKSTQNRFGGPDRLMDFQDVKDDEWTSIGEEMASRL

SEQ ID NO: 8 - protein, 440 aa, synthetic construct
MASELSTSSSILIVGAGTWGCSTALHLARRGYKHVTVLDPYPVPSPIAAGNDVNKIMEHREVAGIIAFATCTRAALKGWQTDPVFKPYFHETGFIQAGHTPALIEHIRQNDLYPSESDFVKLETAEDFRKTMPPGVLTGDFPGWKGWLMKKNAGWIHAKKAMFSAFHEAKRLGVTFITGSPQGKVVSLVYGQDDVTGARTEDGKVHSADRVIVSAGAGTDRILDMENQLRPTAWTLCHIKMTEEEIKSQRYRNLPVLFNIAKGFFMEPDEDKGELKMCDEHPGYVNWVSDPNRPGEKRSIPFAKEQIPREAERRAREFLKDTMPHLADRPLVFARICWDADTPDRFFLIDYHPRYPSLLLACGGSGNGAMQMPSIGGFIADALEGRLQEELKDVCRWRPETAVGRDWKSTQGRFGGPDKVMDFQEVGENEWTRVGKESLL

SEQ ID NO: 9 - protein, 443 aa, synthetic construct
MAGGLGTQSRILILGGGTWGCSTALHLARRGYKNVTVLDAHPIPSPISAGNDVNKIVEQGCFTDGDDEAAVAQTLLHAANEGWQKDPVFQPYYHDTGYIVAGSSPKAIERLVDREVRHQASSFRKLTTAEDFKGTMPTGVLTGDFPGWEGYYKKSGAGWVHAKKALVSAYNEAKRLGVNFITGSPEGKVKSLLLEDGDVRGAITADGVEHRADRTILAMGANAPQLLDFENQLRPTAWTLAHIPMTEEETRLYKNLPVLFNIEKGFFMEPDEDKHELKLCDEHPGYCNWVDQPGSALPQSVPVAKHEVPASAERRMRDFLREIMPHLADRPFTFARMCWCADTRNRAFLITYHPKHPSLVVASGDSGHGFMHIPSIGGFIVDCMENHLQPNFAKSWRWRPETTRDFWGRDVLDRFGAGNKMLDVNETREEGWTNVNATPLTVA

SEQ ID NO: 10 - protein, 447 aa, synthetic construct
MATLELNHTTSILIVGAGTWGCSTALHLARRGYRNVKVLDPHPVPSPIAAGNDINKIMEHKELKSPKPDARSIAFATCTRAALKGWKTDPVFQPYFHETGFIVSGHTPALIKHIETEEIDPSEGDWVALESAEDFRKTMPPGVLTGDFPGWKGWISRVGAGWIHARKAMVSAYNEAQRLGVDFVTGSPQGNVESLIYKDADVVGARTADGLSHYADRTILAAGAGSDRLLDFKKQLRPTAWTLSHIKMTPEEAKKYRNLPVLFNVAKGFFMEPDEEKHELKICDEHPGYCNFVVDPDHQGEKRSIPFAKEQIPLEAEARARDFLRDTMPHLADRPFSFARICWDADTVDRAFLIDRHPEYASLVVAVGGSGNGAMQMPTIGGFISDTLEGKLQKELKDVVRWRPETAIHRDWKSTQNRFGGPDRLMDFQDVKDDEWTKIGEDMASRL

SEQ ID NO: 11 - protein, 447 aa, synthetic construct
MATLELNHASSILIVGAGTWGCSTALHLARRGYKNVKVLDPHPVPSPIAAGNDINKIMEHKELKSPKPDARSIAFATCTRAALKGWKTDPVFQPYFHETGFIVSGHTPALIKHIETEDIDPSEGDWAALESAEDFRKTMPPGVLTGDFPGWKGWISRVGTGWIHARKAMVSAYNEAQRLGVSFVTGSPEGNVESLIYKDGDVVGARTADGLSHYADRTILAAGAGSDRLLDFKKQLRPTAWTLSHIKMTPEEAKKYRNLPVLFNVAKGFFMEPDEEKHELKICDEHPGYCNFVVDPDHQGEKRSIPFAKEQIPLEAEARARDFLRDTMPHLADRPFSFARICWDADTVDRAFLIDRHPEYASLVVAVGGSGNGAMQMPTIGGFISDVLEGKLQKELKDVVRWRPEIAIRRDWKSTQNRFGGPDRLMDFQDVKDDEWTKIGEEMASRL

SEQ ID NO: 12 - protein, 440 aa, synthetic construct
MASELSTSSSILIVGAGTWGCSTALHLARRGYKHVTVLDPYPVPSPIAAGNDVNKIMEHKEVAGIIAFATCTRAALKGWQTDPVFKPYFHETGFIQAGHTPALIKHIRQNDLYPSESDFVKLETAEDFRKTMPPGVLTGDFPGWKGWLMKKNAGWIHARKAMFSAFHEAKRLGVTFITGSPQGKVVSLVYGQDDVTGARTEDGKVHSADRVIVSAGAGTDRILDMENQLRPTAWTLCHIKMTEEEIKSQRYRNLPVLFNIAKGFFMEPDEDKGELKMCDEHPGYVNWVSDPNRPGEKRSIPFAKEQIPREAERRAREFLKDTMPHLADRPLVFARICWDADTPDRFFLIDYHPRYPSLLLACGGSGNGAMQMPSIGGFIADALEGRLQEELKDVCRWRPETAVGRDWKSTQGRFGGPDKVMDFQEVGENEWTKVGKESLL

SEQ ID NO: 13 - protein, 443 aa, synthetic construct
MAGGLGTQSRILILGGGTWGCSTALHLARRGYKNVTVLDAHPIPSPISAGNDVNKIVEQGCFTDGDDEAAVAQTLLHAANEGWQKDPVFQPYYHDTGYIVAGSSPKAIKRLVDREVRHQASSFRKLTTAEDFKKTMPTGVLTGDFPGWEGYYKPSGAGWVHARKALVSAYNEAKRLGVNFITGSPEGKVKSLLLEDGDVRGAITADGVEHRADRTILAMGANAPQLLDFENQLRPTAWTLAHIKMTEEETKLYKNLPVLFNIEKGFFMEPDEDKHELKLCDEHPGYCNWVDQPGSALPQSVPVAKHEVPASAERRMRDFLREIMPHLADRPFTFARMCWCADTRNRAFLITYHPKHPSLVVASGDSGHGFMHIPSIGGFIVDCMENKLQPNFAKSWRWRPETTRDFWGRDVLDRFGAGNKMLDVNETREEGWTKVNATPLTVA

SEQ ID NO: 14 - protein, 447 aa, synthetic construct
MATLELNHTTSILIVGAGTWGCSTALHLARRGYKNVTVLDPHPVPSPIAAGNDINKIMEHKELKSPKPDARSIAFATCTRAALKGWKTDPVFQPYFHETGFIVSGHTPALIEHIKTEEIDPSEGDWVALESAEDFRQTMPPGVLTGDFPGWKGWISRVGAGWIHARKAMVSAYNEAKRLGVDFVTGSPQGNVESLIYEDADVVGARTADGLSHYADRTILAAGAGSDRLLDFKKQLRPTAWTLSHIRMTPEEADKYRNLPVLFNVAKGFFMEPDEEKHELKICDEHPGYCNFVVDPKHQGEVRSIPFAKEQIPLEAEARARDFLRDTMPHLADRPFSFARICWDADTVDRAFLIDRHPEYASLVVAVGGSGNGAMQMPTIGGFISDTLEGKLQKELKDVVRWRPETAIHRDWKSTQNRFGGPDKLMDFQKVGDDEWTRIGEDKASRL

SEQ ID NO: 15 - protein, 447 aa, synthetic construct
MATLELNHASSILIVGAGTWGCSTALHLARRGYKNVTVLDPHPVPSPIAAGNDINKIMEHKELKSPKPDARSIAFATCTRAALKGWKTDPVFQPYFHETGFIVSGHTPALIEHIKTEDIDPSEGDWAALESAEDFRQTMPPGVLTGDFPGWKGWISRVGTGWIHARKAMVSAYNEAKRLGVSFVTGSPEGNVESLIYEDGDVVGARTADGLSHYADRTILAAGAGSDRLLDFKKQLRPTAWTLSHIRMTPEEAEKYRNLPVLFNVAKGFFMEPDEEKHELKICDEHPGYCNFVVDPKHQGEVRSIPFAKEQIPLEAEARARDFLRDTMPHLADRPFSFARICWDADTVDRAFLIDRHPEYASLVVAVGGSGNGAMQMPTIGGFISDVLEGKLQKELKDVVRWRPEIAIRRDWKSTQNRFGGPDKLMDFQKVGDDEWTSIGEEKASRL

SEQ ID NO: 16 - protein, 440 aa, synthetic construct
MASELSTSSSILIVGAGTWGCSTALHLARRGYKHVTVLDPYPVPSPIAAGNDVNKIMEHKEVAGIIAFATCTRAALKGWQTDPVFKPYFHETGFIQAGHTPALIEHIRQNDLYPSESDFVKLETAEDFRKTMPPGVLTGDFPGWKGWLMKKNAGWIHARKAMFSAFHEAKRLGVTFITGSPQGKVVSLVYGQDDVTGARTEDGKVHSADRVIVSAGAGTDRILDMENQLRPTAWTLCHIKMTEEEIKSQRYRNLPVLFNIAKGFFMEPDEDKGELKMCDEHPGYVNWVSDPKRPGEVRSIPFAKEQIPREAERRAREFLKDTMPHLADRPLVFARICWDADTPDRFFLIDYHPRYPSLLLACGGSGNGAMQMPSIGGFIADALEGRLQEELKDVCRWRPETAVGRDWKSTQGRFGGPDKVMDFQKVGENEWTRVGKEKLL

SEQ ID NO: 17 - protein, 443 aa, synthetic construct
MAGGLGTQSRILILGGGTWGCSTALHLARRGYKNVTVLDAHPIPSPISAGNDVNKIVEQGCFTDGDDEAAVAQTLLHAANEGWQKDPVFQPYYHDTGYIVAGSSPKAIERLVDREVRHQASSFRKLTTAEDFKGTMPTGVLTGDFPGWEGYYKPSGAGWVHARKALVSAYNEAKRLGVNFITGSPEGKVKSLLLEDGDVRGAITADGVEHRADRTILAMGANAPQLLDFENQLRPTAWTLAHIPMTEEETRLYKNLPVLFNIEKGFFMEPDEDKHELKLCDEHPGYCNWVDQPKSALPQSVPVAKHEVPASAERRMRDFLREIMPHLADRPFTFARMCWCADTRNRAFLITYHPKHPSLVVASGDSGHGFMHIPSIGGFIVDCMENKLQPNFAKSWRWRPETTRDFWGRDVLDRFGAGNKMLDVNKTREEGWTNVNATKLTVA

SEQ ID NO: 18 - protein, 447 aa, synthetic construct
MATLELNHTTSILIVGAGTWGCSTALHLARRGYKNVTVLDPHPVPSPIAAGNDINKIMEHRELKSPEPDARSIAFATCTRAALKGWKTDPVFQPYFHETGFIVSGHTPALIKHIETEEIDPSEGDWVKLESAEDFRKTMPPGVLTGDFPGWKGWISKVGAGWIHAKKAMVSAYNEAKRLGVDFVTGSPQGNVESLIYEDADVVGARTADGLSHYADRTILAAGAGSDRLLDFKKQLRPTAWTLSHIKMTPEEAKKYRNLPVLFNVAKGFFMEPDEEKHELKICDEHPGYCNFVVDPKHQGEVRSIPFAKEQIPLEAEARARDFLRDTMPHLADRPFSFARICWDADTVDRAFLIDRHPEYASLVVAVGGSGNGAMQMPTIGGFISDTLEGHLQKELKDVVRWRPETAIHRDWKSTQNRFGGPDKLMDFQKVGDDEWTKIGEDKASRL

SEQ ID NO: 19 - protein, 447 aa, synthetic construct
MATLELNHASSILIVGAGTWGCSTALHLARRGYKNVTVLDPHPVPSPIAAGNDINKIMEHRELKSPEPDARSIAFATCTRAALKGWKTDPVFQPYFHETGFIVSGHTPALIKHIETEDIDPSEGDWAKLESAEDFRKTMPPGVLTGDFPGWKGWISKVGTGWIHAKKAMVSAYNEAKRLGVSFVTGSPEGNVESLIYEDGDVVGARTADGLSHYADRTILAAGAGSDRLLDFKKQLRPTAWTLSHIKMTPEEAKKYRNLPVLFNVAKGFFMEPDEEKHELKICDEHPGYCNFVVDPKHQGEVRSIPFAKEQIPLEAEARARDFLRDTMPHLADRPFSFARICWDADTVDRAFLIDRHPEYASLVVAVGGSGNGAMQMPTIGGFISDVLEGHLQKELKDVVRWRPEIAIRRDWKSTQNRFGGPDKLMDFQKVGDDEWTKIGEEKASRL

SEQ ID NO: 20 - protein, 440 aa, synthetic construct
MASELSTSSSILIVGAGTWGCSTALHLARRGYKHVTVLDPYPVPSPIAAGNDVNKIMEHREVAGIIAFATCTRAALKGWQTDPVFKPYFHETGFIQAGHTPALIKHIRQNDLYPSESDFVKLETAEDFRKTMPPGVLTGDFPGWKGWLMKKNAGWIHAKKAMFSAFHEAKRLGVTFITGSPQGKVVSLVYGQDDVTGARTEDGKVHSADRVIVSAGAGTDRILDMENQLRPTAWTLCHIKMTEEEIKSQRYRNLPVLFNIAKGFFMEPDEDKGELKMCDEHPGYVNWVSDPKRPGEVRSIPFAKEQIPREAERRAREFLKDTMPHLADRPLVFARICWDADTPDRFFLIDYHPRYPSLLLACGGSGNGAMQMPSIGGFIADALEGRLQEELKDVCRWRPETAVGRDWKSTQGRFGGPDKVMDFQKVGENEWTKVGKEKLL

SEQ ID NO: 21 - protein, 443 aa, synthetic construct
MAGGLGTQSRILILGGGTWGCSTALHLARRGYKNVTVLDAHPIPSPISAGNDVNKIVEQGCFTDGDDEAAVAQTLLHAANEGWQKDPVFQPYYHDTGYIVAGSSPKAIKRLVDREVRHQASSFRKLTTAEDFKKTMPTGVLTGDFPGWEGYYKKSGAGWVHAKKALVSAYNEAKRLGVNFITGSPEGKVKSLLLEDGDVRGAITADGVEHRADRTILAMGANAPQLLDFENQLRPTAWTLAHIKMTEEETKLYKNLPVLFNIEKGFFMEPDEDKHELKLCDEHPGYCNWVDQPKSALPQSVPVAKHEVPASAERRMRDFLREIMPHLADRPFTFARMCWCADTRNRAFLITYHPKHPSLVVASGDSGHGFMHIPSIGGFIVDCMENHLQPNFAKSWRWRPETTRDFWGRDVLDRFGAGNKMLDVNKTREEGWTKVNATKLTVA

SEQ ID NO: 22 - protein, 445 aa, synthetic construct
MTSSKLTPTSSILIVGAGTWGCSTALHLARRGYKNVTVLDPHPVPSPIAAGNDINKIMEHREVKASETDPWSIAFSTCTRAALKGWKNDPVFQPYFHETGAIVSGHTASLIKHIQEHEIDSSDAEFIKLNTAEDFRKTMPPGILTGNFPGWKGWLNKTGAGWIHAKKAMFSAYTEAKRLGVTFITGSPEGDVVSLIYENGDVVGARTADGTVHRADHTILSAGAGSDRLLDFKKQLRPTAWTLCHIKMTPDEAKKYRNLPVLFNVAKGFFMEPDEDKHELKICDEHPGYCNFVPDPKHGGEVRSIPFAKHQIPLEAEARARDFLRDTMPHLADRPLSFARICWDADTVDRAFLIDRHPEYRSLLLAVGGSGNGAMQMPTIGGFIADALEGNLQKELKHALRWRPEIAAQRDWKDTQNRFGGPNKVMDFQKVGENEWTKIGDKSRL

SEQ ID NO: 23 - protein, 445 aa, synthetic construct
MAPSILSTESSIIVIGAGTWGCSTALHLARRGYKDVTVLDPHPVPSPIAAGNDINKIMEHSELKDGSSDPRSAAFSTFTRAALKAWKTDPVFQPYFHETGFIISGHTPALIDHIRKDEVEPSETNFVKLETAEDFRRTMPPGVLTGDFPGWKGWLHKSGAGWIHAKKAMISAFNEAKRLGVRFVTGSPEGNVVSLVYEDGDVVGARTADGRVHKAHRTILSAGAGSDSLLDFKKQLRPTAWTLCHIKMGPEEVKQYRNLPVLFNIAKGFFMEPDEDKHELKICDEHPGYCNFLPDPNRPGQEKSVPFAKHQIPLEAEARARDFLHDTMPHLADRPLSFARICWDADTPDRAFLIDRHPEHPSLLVAVGGSGNGAMQMPTIGGFIADALESKLQKEVKDIVRWRPETAVDRDWKATQNRFGGPDKIMDFQKVGEDQWTKIGESKGP

SEQ ID NO: 24 - protein, 445 aa, Aspergillus oryzae
MTSSKLTPTSSILIVGAGTWGCSTALHLARRGYKNVTVLDPHPVPSPIAAGNDINKIMEHREVKASETDPWSIAFSTCTRAALKGWKNDPVFQPYFHETGAIVSGHTASLIKHIQEHEIDSSDAEFIKLNTAEDFRKTMPPGILTGNFPGWKGWLNKTGAGWIHAKKAMFSAYTEAKRLGVTFITGSPEGDVVSLIYENGDVVGARTADGTVHRADHTILSAGAGSDRLLDFKKQLRPTAWTLCHIRMTPDEAKKYRNLPVLFNVAKGFFMEPDEDNHELKICDEHPGYCNFVPDPKHGGEVRSIPFAKHQIPLEAEARARDFLRDTMPHLADRPLSFARICWDADTVDRAFLIDRHPEYRSLLLAVGGSGNGAMQMPTIGGFIADALEGNLQKELKHALRWRPEIAAQRDWKDTQNRFGGPNKVMDFQKVGENEWTKIGDKSRL

SEQ ID NO: 25 - protein, 445 aa, Aspergillus fumigatus
MAPSILSTESSIIVIGAGTWGCSTALHLARRGYKDVTVLDPHPVPSPIAAGNDINKIMEHSELKDGSSDPRSAAFSTFTRAALKAWKTDPVFQPYFHETGFIISGHTPALIDHIRKDEVEPSETNFVKLETAEDFRRTMPPGVLTGDFPGWKGWLHKSGAGWIHAKKAMISAFNEAKRLGVRFVTGSPEGNVVSLVYEDGDVVGARTADGRVHKAHRTILSAGAGSDSLLDFKKQLRPTAWTLCHIQMGPEEVKQYRNLPVLFNIAKGFFMEPDEDKHELKICDEHPGYCNFLPDPNRPGQEKSVPFAKHQIPLEAEARARDFLHDTMPHLADRPLSFARICWDADTPDRAFLIDRHPEHPSLLVAVGGSGNGAMQMPTIGGFIADALESKLQKEVKDIVRWRPETAVDRDWRATQNRFGGPDRIMDFQQVGEDQWTKIGESRGP

SEQ ID NO: 26 - protein, 444 aa, Ascosphaera apis
MATPLNKNSKILIVGGGTWGNSTALHLARRGYTDVTVLDPNTMPSAISAGNDVNKIASEGRWLEGDDIDSVHSCVSYLAGKGWLNDPVFKPYYHDTGYVVSASSPEAYERIKKKEIEPGAVKLTTAEDFRKTMPKGVLTGDFPNYTGFWQEKGAGWVHARKAMMSCYNEAKRLGVKYITGSPEGAVISLIDSGSDILGAKTADGKEHRADRTILCAGANANQLLDFKNQLRPTAWTLAHIKMTPEEVKLYKNLPVLFNVEKGFFMEPDEDNHELKMCDEHPGYCNWEPALPGQKWPQSVPVAKHQIPVASERRLRDFLRDIMPQLADRPFCFARVCWCADTRDRGFLISKHPDYPSLVLGSGDAGHGYSMIPVIGSIITDCMEGVMDPRFAKAYRWRPETTQEWWGDELCDRWGAGNKVLDLKKDIAEEGWTNCPQKAAPTSKL

SEQ ID NO: 27 - protein, 446 aa, synthetic construct
MASSNLTLTSSILIVGAGTWGCSTALHLARRGYKNVTVLDPHPVPSPIAAGNDINKIMEHREVRASETDPWSIAFSTCTRAALRGWRTDPVFQPYFHETGAIVSGHTPSLIKHIEEHEIDSSDAEFVRLNTAEDFRKTMPPGILTGNFPGWKGWLNRTGAGWIHARRAMFSAYTEAKRLGVTFITGSPEGDVVSLVYENGDVAGARTADGTIHRAEHTILSAGAGSDRLLDFKKQLRPTAWTLCHIKMTPEEAKKYRNLPVLFNVAKGFFMEPDEDKHELKICDEHPGYCNFIPDPKHGGEVRSIPFAKHQIPLEAEARARDFLRDTMPHLADRPLSFARICWDADTVDRAFLIDRHPEYRSLLLAVGGSGNGAMQMSTIGGFITDALEGHLQRELRHALRWRPEIATERDWKDTQNRFGGPNKVMDFQKVGENEWTKIGDDKCRL

SEQ ID NO: 28 - protein, 446 aa, synthetic construct
MASSNLTLTSSILIVGAGTWGCSTALHLARRGYKNVTVLDPHPVPSPIAAGNDINKIMEHREVKASETDPWSIAFSTCTRAALKGWKTDPVFQPYFHETGAIVSGHTPSLIRHIEEHEIDSSDAEFVKLNTAEDFRRTMPPGILTGNFPGWRGWLNKTGAGWIHAKKAMFSAYTEAKRLGVTFITGSPEGDVVSLVYENGDVAGARTADGTIHRAEHTILSAGAGSDRLLDFKKQLRPTAWTLCHIRMTPEEARRYRNLPVLFNVARGFFMEPDEDRHELKICDEHPGYCNFIPDPKHGGEVRSIPFAKHQIPLEAEARARDFLRDTMPHLADRPLSFARICWDADTVDRAFLIDRHPEYRSLLLAVGGSGNGAMQMSTIGGFITDALEGHLQKELKHALRWRPEIATERDWKDTQNRFGGPNKVMDFQKVGENEWTRIGDDKCRL

SEQ ID NO: 29 - protein, 446 aa, synthetic construct
MASSNLTLTSSILIVGAGTWGCSTALHLARRGYRNVTVLDPHPVPSPIAAGNDINKIMEHREVKASETDPWSIAFSTCTRAALKGWKTDPVFQPYFHETGAIVSGHTPSLIKHIEEHEIDSSDAEFVKLNTAEDFRKTMPPGILTGNFPGWKGWLNKTGAGWIHAKKAMFSAYTEARRLGVTFITGSPEGDVVSLVYENGDVAGARTADGTIHRAEHTILSAGAGSDRLLDFRRQLRPTAWTLCHIKMTPEEAKKYRNLPVLFNVAKGFFMEPDEDKHELKICDEHPGYCNFIPDPRHGGEVRSIPFARHQIPLEAEARARDFLRDTMPHLADRPLSFARICWDADTVDRAFLIDRHPEYRSLLLAVGGSGNGAMQMSTIGGFITDALEGHLQKELKHALRWRPEIATERDWRDTQNRFGGPNRVMDFQRVGENEWTKIGDDRCRL

SEQ ID NO: 30 - protein, 446 aa, synthetic construct
MASSNLTLTSSILIVGAGTWGCSTALHLARRGYRNVKVLDPHPVPSPIAAGNDINKIMEHKEVKASKTDPWSIAFSTCTRAALKGWKTDPVFQPYFHETGAIVSGHTPSLIEHIKEHEIDSSDAEFVALNTAEDFRQTMPPGILTGNFPGWKGWLNRTGAGWIHARKAMFSAYTEAQRLGVTFITGSPEGDVVSLVYKNGDVAGARTADGTIHRAEHTILSAGAGSDRLLDFKKQLRPTAWTLCHIRMTPEEADKYRNLPVLFNVAKGFFMEPDEDKHELKICDEHPGYCNFIPDPDHGGEKRSIPFAKHQIPLEAEARARDFLRDTMPHLADRPLSFARICWDADTVDRAFLIDRHPEYRSLLLAVGGSGNGAMQMSTIGGFITDALEGKLQKELKHALRWRPEIATERDWKDTQNRFGGPNRVMDFQDVKENEWTRIGDDMCRL

SEQ ID NO: 31 - protein, 446 aa, synthetic construct
MASSNLTLTSSILIVGAGTWGCSTALHLARRGYKNVTVLDPHPVPSPIAAGNDINKIMEHREVKASETDPWSIAFSTCTRAALKGWKTDPVFQPYFHETGAIVSGHTPSLIKHIEEHEIDSSDAEFVKLNTAEDFRKTMPPGILTGNFPGWKGWLNKTGAGWIHAKKAMFSAYTEAKRLGVTFITGSPEGDVVSLVYENGDVAGARTADGTIHRAEHTILSAGAGSDRLLDFRRQLRPTAWTLCHIKMTPEEAKKYRNLPVLFNVAKGFFMEPDEDKHELKICDEHPGYCNFIPDPRHGGEVRSIPFAKHQIPLEAEARARDFLRDTMPHLADRPLSFARICWDADTVDRAFLIDRHPEYRSLLLAVGGSGNGAMQMSTIGGFITDALEGHLQKELKHALRWRPEIATERDWKDTQNRFGGPNKVMDFQKVGENEWTKIGDDKCRL

SEQ ID NO: 32 - protein, 446 aa, synthetic construct
MASSNLTLTSSILIVGAGTWGCSTALHLARRGYKNVTVLDPHPVPSPIAAGNDINKIMEHREVKASETDPWSIAFSTCTRAALKGWKTDPVFQPYFHETGAIVSGHTPSLIKHIEEHEIDSSDAEFVKLNTAEDFRKTMPPGILTGNFPGWKGWLNKTGAGWIHAKKAMFSAYTEAKRLGVTFITGSPEGDVVSLVYENGDVAGARTADGTIHRAEHTILSAGAGSDRLLDFKKQLRPTAWTLCHIKMTPEEAKKYRNLPVLFNVAKGFFMEPDEDKHELKICDEHPGYCNFIPDPKHGGEVRSIPFARHQIPLEAEARARDFLRDTMPHLADRPLSFARICWDADTVDRAFLIDRHPEYRSLLLAVGGSGNGAMQMSTIGGFITDALEGHLQKELKHALRWRPEIATERDWRDTQNRFGGPNKVMDFQKVGENEWTKIGDDKCRL

SEQ ID NO: 33 - protein, 446 aa, synthetic construct
MASSNLTLTSSILIVGAGTWGCSTALHLARRGYKNVTVLDPHPVPSPIAAGNDINKIMEHREVKASETDPWSIAFSTCTRAALKGWKTDPVFQPYFHETGAIVSGHTPSLIKHIEEHEIDSSDAEFVKLNTAEDFRKTMPPGILTGNFPGWKGWLNKTGAGWIHAKKAMFSAYTEAKRLGVTFITGSPEGDVVSLVYENGDVAGARTADGTIHRAEHTILSAGAGSDRLLDFKKQLRPTAWTLCHIKMTPEEAKKYRNLPVLFNVAKGFFMEPDEDKHELKICDEHPGYCNFIPDPKHGGEVRSIPFAKHQIPLEAEARARDFLRDTMPHLADRPLSFARICWDADTVDRAFLIDRHPEYRSLLLAVGGSGNGAMQMSTIGGFITDALEGHLQKELKHALRWRPEIATERDWKDTQNRFGGPNRVMDFQRVGENEWTKIGDDRCRL

SEQ ID NO: 34 - protein, 446 aa, synthetic construct
MASSNLTLTSSILIVGAGTWGCSTALHLARRGYRNVTVLDPHPVPSPIAAGNDINKIMEHREVKASETDPWSIAFSTCTRAALKGWKTDPVFQPYFHETGAIVSGHTPSLIKHIEEHEIDSSDAEFVKLNTAEDFRKTMPPGILTGNFPGWKGWLNKTGAGWIHAKKAMFSAYTEARRLGVTFITGSPEGDVVSLVYENGDVAGARTADGTIHRAEHTILSAGAGSDRLLDFKKQLRPTAWTLCHIKMTPEEAKKYRNLPVLFNVAKGFFMEPDEDKHELKICDEHPGYCNFIPDPKHGGEVRSIPFAKHQIPLEAEARARDFLRDTMPHLADRPLSFARICWDADTVDRAFLIDRHPEYRSLLLAVGGSGNGAMQMSTIGGFITDALEGHLQKELKHALRWRPEIATERDWKDTQNRFGGPNKVMDFQKVGENEWTKIGDDKCRL

SEQ ID NO: 35 - protein, 446 aa, synthetic construct
MASSNLTLTSSILIVGAGTWGCSTALHLARRGYKNVTVLDPHPVPSPIAAGNDINKIMEHREVKASETDPWSIAFSTCTRAALKGWKTDPVFQPYFHETGAIVSGHTPSLIKHIEEHEIDSSDAEFVKLNTAEDFRKTMPPGILTGNFPGWKGWLNKTGAGWIHAKKAMFSAYTEAKRLGVTFITGSPEGDVVSLVYENGDVAGARTADGTIHRAEHTILSAGAGSDRLLDFKKQLRPTAWTLCHIRMTPEEAKKYRNLPVLFNVAKGFFMEPDEDRHELKICDEHPGYCNFIPDPKHGGEVRSIPFAKHQIPLEAEARARDFLRDTMPHLADRPLSFARICWDADTVDRAFLIDRHPEYRSLLLAVGGSGNGAMQMSTIGGFITDALEGHLQKELKHALRWRPEIATERDWKDTQNRFGGPNKVMDFQKVGENEWTKIGDDKCRL